European Patent Application EP 4 488 371 A2, published January 8, 2025. Title: COMPOUNDS AND METHODS FOR MODULATING ANGIOTENSINOGEN EXPRESSION. Applicant: Ionis Pharmaceuticals, Inc. The sequence listing filed with the application follows.

SEQUENCE LISTING (36 sequences)

SEQ ID NO: 1 - RNA, 2587 nt, Homo sapiens
  source 1..2587: mol_type = mRNA
atcccatgagcgggcagcagggtcagaagtggcccccgtgttgcctaagcaagactctcccctgccctctgccctctgcacctccggcctgcatgtccctgtggcctcttgggggtacatctcccggggctgggtcagaaggcctgggtggttggcctcaggctgtcacacacctagggagatgctcccgtttctgggaaccttggccccgactcctgcaaacttcggtaaatgtgtaactcgaccctgcaccggctcactctgttcagcagtgaaactctgcatcgatcactaagacttcctggaagaggtcccagcgtgagtgtcgcttctggcatctgtccttctggccagcctgtggtctggccaagtgatgtaaccctcctctccagcctgtgcacaggcagcctgggaacagctccatccccacccctcagctataaatagggcatcgtgacccggccgggggaagaagctgccgttgttctgggtactacagcagaagggtatgcggaagcgagcaccccagtctgagatggctcctgccggtgtgagcctgagggccaccatcctctgcctcctggcctgggctggcctggctgcaggtgaccgggtgtacatacaccccttccacctcgtcatccacaatgagagtacctgtgagcagctggcaaaggccaatgccgggaagcccaaagaccccaccttcatacctgctccaattcaggccaagacatcccctgtggatgaaaaggccctacaggaccagctggtgctagtcgctgcaaaacttgacaccgaagacaagttgagggccgcaatggtcgggatgctggccaacttcttgggcttccgtatatatggcatgcacagtgagctatggggcgtggtccatggggccaccgtcctctccccaacggctgtctttggcaccctggcctctctctatctgggagccttggaccacacagctgacaggctacaggcaatcctgggtgttccttggaaggacaagaactgcacctcccggctggatgcgcacaaggtcctgtctgccctgcaggctgtacagggcctgctagtggcccagggcagggctgatagccaggcccagctgctgctgtccacggtggtgggcgtgttcacagccccaggcctgcacctgaagcagccgtttgtgcagggcctggctctctatacccctgtggtcctcccacgctctctggacttcacagaactggatgttgctgctgagaagattgacaggttcatgcaggctgtgacaggatggaagactggctgctccctgatgggagccagtgtggacagcaccctggctttcaacacctacgtccacttccaagggaagatgaagggcttctccctgctggccgagccccaggagttctgggtggacaacagcacctcagtgtctgttcccatgctctctggcatgggcaccttccagcactggagtgacatccaggacaacttctcggtgactcaagtgcccttcactgagagcgcctgcctgctgctgatccagcctcactatgcctctgacctggacaaggtggagggtctcactttccagcaaaactccctcaactggatgaagaaactatctccccggaccatccacctgaccatgccccaactggtgctgcaaggatcttatgacctgcaggacctgctcgcccaggctgagctgcccgccattctgcacaccgagctgaacctgcaaaaattgagcaatgaccgcatcagggtgggggaggtgctgaacagcattttttttgagcttgaagcggatgagagagagcccacagagtctacccaacagcttaacaagcctgaggtcttggaggtgaccctgaaccgcccattcctgtttgctgtgtatgatcaaagcgccactgccctgcacttcctgggccgcgtggccaacccgctgagcacagcatgaggccagggccccagaacacagtgcctggcaaggcctctgcccctggcctttgaggcaaaggccagcagcagataacaaccccggacaaatcagcgatgtgtcacccccagtctcccaccttttcttctaatgagtcgactttgagctggaaagcagccgtttctccttggtctaagtgtgctgcatggagtgagcagtagaagcctgcagcggcacaaatgcacctcccagtttgctgggtttattttagagaatgggggtggggaggcaagaaccagtgtttagcgcgggactactgttccaaaaagaattccaaccgaccagcttgtttgtgaaacaaaaaagtgttcccttttcaagttgagaacaaaaattgggttttaaaattaaagtatacatttttgcattgccttcggtttgtatttagtgtcttgaatgtaagaacatgacctccgtgtagtgtctgtaataccttagttttttccacagatgcttgtgatttttgaacaatacgtgaaagatgcaagcacctgaatttctgtttgaatgcggaaccatagctggttatttctcccttgtgttagtaataaacgtcttgccacaataagcctccaaaaaaaa

SEQ ID NO: 2 - DNA, 18000 bp, Homo sapiens
  source 1..18000: mol_type = genomic DNA
cagagcaagaccccaactctaaaacaacacacaaaaatacagccatttctcctgggtgaaatgggggagctcagactattttgttttatttgtcaggagtctaaagcccatgtgagccaacttaagaaaattctgtttgtatttgagtgttctttattggaaagaaatggacttttccctaatgagcccattttacaaatcgagagctccaaatgcccggttccagcccccatgatatagatgggcagcaatgaggaccagaaatgctgggaagtgtccttgtcatgcaaggaaaacttggaacttcaaggatccatcatgggatgcaggacagtaggctccacccctcttcctgctttccagtaaatgatgttcagggctcacatgcctcttccaaggcatgatgtggggttgcagttctgatcccagcagagaacaaggctcctgtgaaacaattagttttggctcagaggcaaaaaatggaaaccccattcctgtatttacccttcattctttccttacctcatacagctggttccaggtttgattgcatcatatacataaataaataatctgctttcctggtttggtttagttttgctggagagaggagtttatgtgttcatcccatgactagctgggtggtcaagagattggaaagtaggagttctagtttagaccaagtctcatctcagaaaccacagagtagaactgatcccaaacgtcatcatccctgtagggaaaagaaagagagatcagactgttactgtgtctatatagaaagggaagacataagagactccattttgaaaaagagctatactttaaacaattgctttgctgagatgttgttaatttgtagctttgccccagccactttgacccaacctggagctcacaaaaacatgtgttgtataaaatcaaggtttaagggatctagggctgtgtcaaagtggctggggcaaagctacaaattaacaacatctcagcaaagcaattgtttaaagtacagctctttttcaaaatggagtctcttatgtcttccctttctatatagacacagtaacagtctgatctctcttttttttccctacatatcccaatagcacctgcctgactaatacatcatgctctgctgactccatatgtggctggtttcctggatccgattctgactgatggtatctgttctcacgctgctaataaagacataccagagactgggtaatttataaagaaaaagaggtttaatggacttatgtgttccacgtggctggggaggcctcacaatcatggtggaaggtgaaggaggagcaaaagcacatcttacatggtggctggcaaaagagagaaagcatgttcaggggaactcccctttataaaaccatcagatctcatgagacttatgcactatcacaagaacagcatcagaaagatccaccctcatgattcaattacctcccactgggtccctcccatgacacatgggaattatgggagctacaattggagatttgggtggggacacagccaaaccatatcagatggcttatttggtttctatgtagaacctctgcttttcattcaacagtcttcatttagccacagataagctctgtccctaacttccactgatggaatgtacacataagaaacttccactgatggaatgaacacagaaggtgcctactgggaagaaaactggcctgaatctgagctgggtcaaatgtctgcagtcagtttgaatggctgctccttatgggaataatttacattctcaataaaattctctagcaattttctgattgattttaatgagctttaaagccttacgtagaagatcccccagctgatagtcagccttgggcatggattaagggcttttaaccaatcttgcaacaagtttaagcagatattctttattgggtccaatctaaccaaaattattttcttatgttctccccagtaacgtgtcattattaagagaagtttggcttgcttagaggccaaatttagagggtcctgaaattttattttcttttacaccactttccagcatgttacctgatcagttgtttattatctttgctgttgaatggagtgatcattccaagggcccgaggcaggaggcccaggcacagtggaaactctcccaaagaccaggatctttgttttgttccctgacatatgctgagcaccaggaatagtgagtgaatgaaacaaattgtgaggctttaaagagccgaaatatttaaacactgggcacaaggttgttgcttaatcagtgctagatccttacctcccccttgtgtccaggtggacttgttactgcagttaaaccacttgctgatcctcaaacaactagttagtggcacagccaggcctaggaccccagtctctactgttccaactaacccattcgcaggcaggagcactttgaatggtctcttattttaaaaaaattaaattaaaattgtctatttatttagagacagagtcttactctgtagcccaggctcgagtgcagtggtgcaatcatagctcactgtaacctccatctcctggcctcaaaaagtgtttgaattacagatgcgaggcactgtacctggcccgaatgttctgttcagacaaagccacctctaagtcgctgtggggccccagacaagtgatttttgaggagtccctatctataggaacaaagtaattaaaaaaatgtatttcagaatttacaggcccatgtgagatatgatttttttaaatgaagatttagagtaatgggtaaaaaagaggtatttgtgtgtttgttgattgttcagtcagtgaatgtacagcttctgcctcatatccaggcaccatctcttcctgctctttgttgttaaatgttccattcctgggtaatttcatgtctgccatcgtggatatgccgtggctccttgaacctgcttgtgttgaagcaggatcttccttcctgtcccttcagtgccctaataccatgtatttaaggctggacacatcaccactcccaacctgcctcacccactgcgtcacttgtgatcactggcttctggcgactctcaccaaggtctctgtcatgccctgttataatgactacaaaagcaagtcttacctataggaaaataagaattataacccttttactggtcatgtgaaacttaccatttgcaatttgtacagcataaacacagaacagcacatctttcaatgcctgcatcctgaaggcattttgtttgtgtctttcaatctggctgtgctattgttggtgtttaacagtctccccagctacactggaaacttccagaaggcacttttcacttgcttgtgtgttttccccagtgtctattagaggcctttgcacagggtaggctctttggagcagctgaaggtcacacatcccatgagcgggcagcagggtcagaagtggcccccgtgttgcctaagcaagactctcccctgccctctgccctctgcacctccggcctgcatgtccctgtggcctcttgggggtacatctcccggggctgggtcagaaggcctgggtggttggcctcaggctgtcacacacctagggagatgctcccgtttctgggaaccttggccccgactcctgcaaacttcggtaaatgtgtaactcgaccctgcaccggctcactctgttcagcagtgaaactctgcatcgatcactaagacttcctggaagaggtcccagcgtgagtgtcgcttctggcatctgtccttctggccagcctgtggtctggccaagtgatgtaaccctcctctccagcctgtgcacaggcagcctgggaacagctccatccccacccctcagctataaatagggcatcgtgacccggccgggggaagaagctgccgttgttctgggtactacagcagaaggtaagccgggggccccctcagctccttctcggtcttgtctctctcagatgtaactgagctgtgggctaggaggaaaaggccgggaggaggcacggtgatgactgaaaaacctctcccctctcataagaccagtcatccggacgcgggctttcccccactcggtgcccacctggggtcttacaggaggagctgctcctcctcagcaataggacaagatggtcaggtcttcctgcttccgctgagaaaagttagggtcctcaggaacggagcagactggtacaggaacagagtcatcatggccaagagtccaccgggtcctcttgccatcaggaggaatagcagggcttgtgcaggaattggggctggagggaagggccgggctcggtcagtctccagctgggatccccagagtggtcaccctacccctccctcgagacagactgcctgactgtgtgtcatcaggctggtcaccatctccctgaacctcgatttgctcacctataaaatggaactaataacgatgcctgggctccctgtctcaggggctctggtatagctgaagagaactaatataacatgaaagtgctttctaagctttgggataagctaaaaggcagattccaattttattcgagggcagcgtagattggtgcttcagctcgtggatgacagagtcagggggcctggttctgagtcctagttctgtctcttcccagctgtgtgacgttgaacaagtcactggacctctctgttcctctgcaaaacagcatgaaccaattcattaactacttctccaggatgcagtaggtcccagggactatcctaggaatgtgggctgtattagtaaacacaacagcgggaaccctgttccggggctcacattcacatcagagcaaacagacaaagacgctggacagaataagtgcataactacatggtacagagggttataaggagggaaaaggggagctggatgagagagttgagagtgcccggtgtggtggggaaagctgcagggtgaaatactgcatcagggaaacctcagggaaggtgaggactatggtgaggtcagaggggttgatatgagaacagtgccctgcaaatggcaggcaccacaggagcatgagccgtcatcttcacctttagcattcagcccgggagaagtagggagacatagaaggggcaggtgctggccaagaggcaggggcaggagaggagaaggcggaggggcactcagggcgagggtgtcaggcccgccaccccagagcaccattactcccaggacgcggctgcgtgcagacctggaaccagcctagggagcagccgcagatcacaactgagaacaaacgacagtctctgcctcaaaaatggcccatggaattgcgtctctggagacgctgcctgagcaggagcagcacagtgagcgggctgcatcgaccagcgccatccaaaccccgaacagttggcgcttgtcaggcaggacttcccagcagtcggttcccacaggtttcccctgttgacctgatttgatgtgactgtctagattaggtgtgaactggtggcttaggcttctctgcacagaaaggcctgcaagcagcagagagagttttctgttccatttttccatgtcatgtggctcttcctgagaacagcggatggagtcaaatgcatggggagtggggtgagatggtagctgaggtcagaatttggcatttgaatgactgaagcagaacaaaacacaccaggtacttcagcagctgcaccgtgttgagggcaggtgctggttacgggtctgggtgagggaagccagctgccaatgtaagaagaatgactgggtatgcttagatgaagcagaaaaatctaggcatcaaggtggccttgagtcagtgatgacacgctacagctccaaggaagcctggcctagccctggggggacagaaaaggccaagaagtgacgatattgcagtacacccccctccacaagaaatgagtgagatgtggtacaaaatgttagaattgaatgaatcaatagaataaacgttcatcccttcaatcaagaagagtcagatgaaatgaattagcagggccagcccaagaacctcttctgggggtctcagggtagctttcatttgtagcagctgaggctgaagcccagctgcaaggcctttgagagaacgtggtgctggacccgtgtctagggcaggggttctaaaccctgcttacatatcagagtcacctgagaattttctatttttttttttttttttttatacgtggtcccagcacagactaaggaatccaactatcattgggcaagccatgctaggtatgcatgcctttggggctctgcaggggatagcgctatgcagggatggttgagagctggttttggggttgagacacgtgggaaatacttggactttgggctgagcctgtggtgctcaatcccggctgcatgttgggaccacagggagatgacaaaaccatccccagccctcaccctagggccctcgaatgagcatctcaggggtctaggaggcctccacaaagacctactgattggcacacacttgtttctctaggaagagaacttacagctgcaggcaggagcatgtcttaatctgcttgggctgccataagtaccacagactgggagggtttaacaacagaaatgtgttatctcacagttctggaagctagaagcctgggagccagccatcagcagagttggtttcctctgggtcctctatccttggcttgtagatggccgtcttctctctgtgtccccacatggtcttccctctgtgtccccacatggtcttccctctgtgtgtgtccatgtcctcatctcctcttctcataaggacacaggtcatattagatcagggctcaccctcatggcctcattttaacttaatcatctctttaaagatcctgtctccaaataatggtcacattctgaggtcctggggttgaggacttcaacacgggcattatggccgttgggggaggtaggacataattcagctgatattggtgcattttgcacttggatcatgtagatattttccatggagctttgaatccatttcttcttttttttgtagacatgaatggatttattctgggctaaatggtgacagggaatattgagacaatgaaagatctggttagatggcacttaaaggtcagttaataaccacctttcaccctttgcaaaatgatatttcagggtatgcggaagcgagcaccccagtctgagatggctcctgccggtgtgagcctgagggccaccatcctctgcctcctggcctgggctggcctggctgcaggtgaccgggtgtacatacaccccttccacctcgtcatccacaatgagagtacctgtgagcagctggcaaaggccaatgccgggaagcccaaagaccccaccttcatacctgctccaattcaggccaagacatcccctgtggatgaaaaggccctacaggaccagctggtgctagtcgctgcaaaacttgacaccgaagacaagttgagggccgcaatggtcgggatgctggccaacttcttgggcttccgtatatatggcatgcacagtgagctatggggcgtggtccatggggccaccgtcctctccccaacggctgtctttggcaccctggcctctctctatctgggagccttggaccacacagctgacaggctacaggcaatcctgggtgttccttggaaggacaagaactgcacctcccggctggatgcgcacaaggtcctgtctgccctgcaggctgtacagggcctgctagtggcccagggcagggctgatagccaggcccagctgctgctgtccacggtggtgggcgtgttcacagccccaggcctgcacctgaagcagccgtttgtgcagggcctggctctctatacccctgtggtcctcccacgctctctggacttcacagaactggatgttgctgctgagaagattgacaggttcatgcaggctgtgacaggatggaagactggctgctccctgatgggagccagtgtggacagcaccctggctttcaacacctacgtccacttccaaggtaaggcaaacctctctgctggctctggccctaggacttagtatccaatgtgtagctgagatcagccagtcaggccttggagatgggcagggggcagccctgcggacatacctggtgaccacccttgagaagtggggaagtggctgctccgctgggtccctggatgggccgtccacctcctggacctgctgccctactatgtgcacgactatacaacatcctttttcttacatcatttaatccccttatgatgtggtgaagaggtatttgtgcctttgtttaccagtgaagaaatagagactcggagaaacaaagtgccttgctcaagatggcacagccaccagtgggggtcctgggattgaaacccacatctcctggccccacagcccagttctacactcagaagggtcaggttcatatctcttgagaaggtcaggaactggggtccctggcccatgcagaaataagcaattggcttgcttaaatccctttcatgttaggaggggcattactgaaaaccctctactacaaagattgttgatttttttttttttttttattgagacagggtcttgttctgtcacccaggctgcagtgtagtggtgccatcattgctcactgtagccttgaactcctggcctcaagcgatcctcccacctctgccttccaaagtgttgggattaaaggtgtgagccactgcacccagccacagattgcttaaagcattcatttaacaaatacttgttgaggatttgctacttgtaagactttaagcctggcatctcagaggaggccagaggagggctgtataggccctgcctccaggcttttaaaggtcaatgggcaaatgcctaggatttggagctgcagggaaacgtgctccacaaggtaactcagggaagcctcggggctctcagaggacagaggtcactggggagcggagagcaggccttgcctggcagtgagggcaacagggctggtgaagctaggagcaagcatgatgagcccagcctgcagagtttggggcaaggaacgaggatggggcggttggcttggcatgagtgttgaaccagaaaatgggcctggggagggcagagctggagacactttgaacgccatgcttggtaggtgtgggaatggggacgcgttctgttcagaggtcatcccggaagcctgccgtgtgcagactggaggcagggaggattgtttgaaggttacgcaagagtccaggcacacagtcacgggaacacgtgctcagggagcagctcggcaaatccatgggtggggtggggctgaggggtgtgtctaagagacactgaggaggctctgtcaagatgttaacctcgtgagggacagagagccaggcgggaggtgaaagacaagactgtggagaaagaggttcagtggcgcatagtgatttttcttaccacaacaacctccttgaggtctttcccttcgggttcagggagaggtgatagatggggggattgctcagccctggcactgactggtcacaggggcagaggccagcccgagggttgcccggttgagggtggcagcacactgtgcagggcagagcagggacacatggacttagcctgctgtccctaggagaagtgctgggaggagcgctcactgagaaggagggtcctgcagaaggcaaaggcaagaaagccagtggcatctgaaatgggtctcccttcgaaagagagcacatccacctgacccagaccgcagagccaggccaggaggaagaggaggaagaataaaaaagccaaccacatcgggactcaaaggaagcccaggatcctcgccggcctccaccgcatgctgccctgaccctgccccacttcctaactttgctggcctcagtttccgtcaaaggaggcagccacttcctgcccacatggtctgtccagtgaggagatcgggggctgtctcgggacctctaggtttccctttagcaatgatgttctatttacatgacctcagcaggcagctagatgtgtcccactagagaggacctgaggatctggggcctgatgggctccagggtaccgtctgcccagtgcttgctgtgctcctgagcatggggcgctggccctggtggtttccatgacaccaggtcctgacttgacctcgacagatttacctagcctccggatgagaatggtgagctgtgcatgtcagacgagcagagggaagacggcagccactctcatgtcaaatcccagcgtcttttgggaggcagcttcccttttttagtttagtttgttggaagaaaagaattgtccctttcccccctctaaactaaaagccttgccagcccaggtgggcagcaccgaggtccctgcagggaacgtgcaaggggaaccctgcagtttcccgctcacatgcccttccgagactgagtgctccgaggactgaggacgagaaatatgccaggtctgccactgccttcttacgagacccggacccaggggaggcacagccatgcccagctcctgcctgccagttctgtcctcccagctgccctactttcatgctgggacctccaattcagtacaaagggagacctcactgtttctgaaccatctctactcagactcccaagtgccacgtgcccaggggactgttctgtgacaaacttatacacaacttcaccctattctcctaagaacaaccgcagaataggcctttcaggatgagtgggaggacagccgagggcagggatgtgctagtgtaaggtcgaggcagagggtgggctgctgtcatggaaagaccccaggtaactgcgtcacacacaaatttgtgtccttctcccacaacgggctctcccgagttctctgtcatctgcacggccctgtgagcaggaggggaaacagagggctcacccctgcccccaaggcccagtgtgcaaatccattcatcacaacgaggttgtgtgagtctccccagtagcaagggctgctgaggaatggagccctcgtttccggggcctgcgtggcccactctgtattctatgactgtgatgggggagggtgggggccacaggacagctggtgggctctgccatggctggggctagacatggattaaaaagtgagtatgagcaggggcctctaggagtggtgggatagtgcggtggtggccacatgtcattctacgtgcgtccaaacctacagaatgtaaaacaccaggagggagactcaaagaaaactatcaactttgagtgctgaggacgtgtcagtgtaggttcgtcagttgcaacaaatgggccacgctggtgtgagatgttgatcacgggggaggctgtgtagtgggggacaagagttatatgggaactttctgtactttctgctcgattttgctgtgaacctaaagtcactctaaaaaataacatctcttaaattttttaaaaagtgagtgtgtcaaaccacagcctttgggtcaggacagttctaggtttgagttgacctggcaggtaccagtggcttatgtcccttaaggtgacagatgcaaaacccccggtttggtgcctggcatgttgtgtgtcttgcaggtggcggttagggctgcctcagtgaactcaaatggctgcattttacaggagaaatatttgagccacacttgcggtcctgtggccaggagaatgcagagtggcctggggggggccaaggaaggaggctgaggcagggcgaggggcaggatctgggcctttggtgtctgccagccctcattcctgcccctgtcttgggtgactcttccctccctgtctcctgtctggatttcagggaagatgaagggcttctccctgctggccgagccccaggagttctgggtggacaacagcacctcagtgtctgttcccatgctctctggcatgggcaccttccagcactggagtgacatccaggacaacttctcggtgactcaagtgcccttcactgagagcgcctgcctgctgctgatccagcctcactatgcctctgacctggacaaggtggagggtctcactttccagcaaaactccctcaactggatgaagaaactatctccccggtaggagcctcccggtctcccctggaatgtgggagccacactgtcctgcccaggctgggggcggggtggggagtagacacacctgagctgagccttgggtgcagagcagggcagggccgcggtggcacggggctgggcaggcggcctgtgtgtctgtctaccagtcctctatccagccagcacccagctctccagttagtgtctgtctttcaagtgcaggcaaggtaaaggaggagaggaagaatgctttttctacacttacacttgcctggtagttttggagggggagaaaacattgcaatccgccctctgagagaggaccattttggtcccacacctgacacacagcacacctgtgacatccaagagcttcttggaactgacttgccaggagggttcggacttcgcgtgagcgggggtggggccttctcagggagcgtcccttgactccagaacgcccttgctggcggctggcggctgggtggggataggtgttgttagctcctctttcctgctgcaattcctttccacagagccctggactcaaactacacatcaccccagatcatcgaggcctggaaatctgctcccagaggcaggcattgagtgacacgatggcttgacatcaactctgggtgttttttatgttttaaaaattgtgatggtaaaatatacgtaacaaaatttgccatcgtaaccattttcgagtgcacagttcagtggtactaggcccattcacactgttgtgcagccatcacccccgtccatctccatttatcttctcaacttcccaaactgaagctctgtcctgctgaaacactaactctccatttccccttccccttggccccggcaaccaccacgatgtcctcgaggttcacccatgttgtagcacatgtcagaatgtccttccttttgaaggctgaataatattccattgcatgtggttaccaccttttgtgtatccactcatccatcgatggacacgtgggttgcttccacctttgagctgctgtgaatagtgcagtgtaccctgtaaacatgggtgtactgtcagctcttataagtgcttgatacatcactggaaatgtccatgggctctgaaggatgccaaaagatggaagaggctctatacgaagatcaatcgagttgacatagcaacgtgtccagcacgaggttgacactgtaccctcctgcctctctccttttcatgggtgtcatgtcatcaagaacactgctgtggcagtagtaagacacagtgcattatttcagagaatagcatttaaaaattacccaagtaacacaccttcaatgcagccaacctaaaaacagaatgcaccaaaggacaaccattcctaggtcctcatcggtaaatcttctatgtccctcacatagtattgcaaatgacatgaaggatttttattgtaggttttgctgaaattttccccaagggggaggatgacttagttgggtgatggggggagcaaacatccctgtcgtcagggttgggtgcaaggagcataagcctgcctggcctctgggagagccctcactgtgtggcctggagccttcctaactgtgcatcatctccccaggaccatccacctgaccatgccccaactggtgctgcaaggatcttatgacctgcaggacctgctcgcccaggctgagctgcccgccattctgcacaccgagctgaacctgcaaaaattgagcaatgaccgcatcagggtgggggaggtatgtgtgagcctgtgtctgtgcctgacctgggttccaagtgtgcacagggtgggaggcatggatgtaagggacacagaggaggctatgggtggggccagcagggcaagagggagcggagagtagggccaaaggtgggagagaagtagccagagcattctggggccttccaggtgcagagcagcaaatccctccccatccctgctgtgcctcctcctgctaggtgtgtgttccatggtcctgcttggccttgccttgcctcagggtcctccagggttcctatagtggagttgaaaccgggatgaagacagcaagcacccctggacctggtgccctgggcccagccccttcttcagggaaatgctgagcagcagacagaatgtccccctgccatgtggcaccatgcacatctgcagctaccaaggatgtgccttgatgttctgggccctgtgctcagtgctggggagaaagtgggagttcttacgggggccagcgggaagagccctctgtgctaagttagctaagccctggcactggtgggccatggccaagggagccaggaattctgcctgggacatcagggcagaatgtgaagatgggaggatgtaaggggtgtgttagggaggagccggcatgtgagtttggccattgtggccaattaacggtcatctacacacagacacacccttgcctacactgaggggcaggcatacactgtgcatcctcctggcaggctggaaaatgtccccctccaggacagtgcacagcacagaggtcctgagcccaccccggccctctagccctcagcaccctgggtcacccagtgcgccctcagaatgatcctgatgtctgctgctttgcaggtgctgaacagcattttttttgagcttgaagcggatgagagagagcccacagagtctacccaacagcttaacaagcctgaggtcttggaggtgaccctgaaccgcccattcctgtttgctgtgtatgatcaaagcgccactgccctgcacttcctgggccgcgtggccaacccgctgagcacagcatgaggccagggccccagaacacagtgcctggcaaggcctctgcccctggcctttgaggcaaaggccagcagcagataacaaccccggacaaatcagcgatgtgtcacccccagtctcccaccttttcttctaatgagtcgactttgagctggaaagcagccgtttctccttggtctaagtgtgctgcatggagtgagcagtagaagcctgcagcggcacaaatgcacctcccagtttgctgggtttattttagagaatgggggtggggaggcaagaaccagtgtttagcgcgggactactgttccaaaaagaattccaaccgaccagcttgtttgtgaaacaaaaaagtgttcccttttcaagttgagaacaaaaattgggttttaaaattaaagtatacatttttgcattgccttcggtttgtatttagtgtcttgaatgtaagaacatgacctccgtgtagtgtctgtaataccttagttttttccacagatgcttgtgatttttgaacaatacgtgaaagatgcaagcacctgaatttctgtttgaatgcggaaccatagctggttatttctcccttgtgttagtaataaacgtcttgccacaataagcctccaaaaattttatctttcatttagcagccaaacagatgtatacaattcagcagatagactgtgcaaacgaaagtgctttcctggactttggatggaatttccatgggaggtctgagccagtacttagcagtcctttgaagttttaggtgatgcttttctctggacacttccattggtaagcagtggtggccatctgtgtgatggacagggggcgggaagagggtgacagggaaggccccataccccatgtggcacctgggaaaggaaccaggcagatgggacttcttccgtcctggtgacacagggccagactgctgctggtattgtgccccgggagtggaaggtagagaaataaatcttcacaaataaatatttgcaattttcccccatctgttgagtgcctctgcctgctcctcctcgatgggattaggcccacagttcggaatcttggggagagccaaggaagcggtaggcacccagtaggcccacggccgtcggctgatagcaatggtgatgctgtcctacctacttgtgtaaggcattcgatcttcctcccttccatacatattgaaataaataagccgcgcaatgtgttagctattgatcagaactaaagtgaagtcagccacggggattacaaatctcggcttctcccctcatgttcctgagagtcttcccctggttttgaacacatctccctagctcgatgtcaaggtgagggattctgtcggcaacagcagtgcccttagttgcttcgtcgtaactccccgtcaccggttttattcagttaccttccagtcccactctcagagcttcctggcttgttctgctctcaaagcgggtagagctggcacacatggactctccgaaacggctgcaagatgccaagtttctcggaagaactggaagcacagagaccagaagtgccttaaggtctcgctattcagtgtggcgcttagaccggcagtggcggcagctgccctgggagcttgttagaatgtggcttctcacgcccctcctggacctacagagtcagaatctgcagttttacaggaggtccaggcttggaagttgctcgtagagacctgagacagcgcagccacgtgctggaaacaaagcatttaagtttgtgactttattttaaaaggcagcaggcagtcgacaaaccaatttcttctacttagaggcggcttcggcttctggaagtcgctaggagtataaagttgccaaccagcgctgttctcccgctgttttctgtgcacttataaatgggaagttaggtcaggatagatctctcagctattacaaggatacaaaatacgaacattctacaagttacttaacacacacacacacacacacacacacacacacacacacaaaattaattccacaggtcagtttctctgaaacattttttcactaaattctaagtcttcctggagttgcaagtgcctatctcctagacaaggcaattactcaccaactaaaatcactgtcaatctgagatttcggctgggcatgagaccatggtcaggggatgctttgaacagcctctgaggaaattagtgagtttgaaaaatggaaagatttttattactcacttggcagtaaaacctgatggggacagacgtcaggctgtttaagatcctcagaagaaaaagttgatagtgtgaatattcctaaatttgccacacgaagatgtacatgtgattataaggtgctgttgcagaagcccctgggggtgttatgggatatacactatatgggccactttaccttcctaaaatctgaaaaacttcaactactgaaacatggactgaaggttttgaatagtggatggtgaatttgaataccatcccgtgtgatttttttttctagcagactttagttttttagagcagttttaagcccacaccaaaactgagaggaagatacagcaatttctcatataccccctactaccttccagtctcccccattattgacatcccccacccagagtggtccatttcttacaacccacgaacctacattgacacatcattattactcaacgtccatagtttacattagggttggctcttggtgttgtacattctatgggtttagacaattttcaggagtttcactgacctgaaaatcctctgtgtccctcctattcacccctccttccctcctaaccactggtaaccaccgatcctattcccatcttctccatagttttgcctttcccacccaggatgtcatatagtggaatcattcagtatgtggcctttccagattagcctctttcacttagtaatgtgcatttaagtttcctccatgtcttttcatgatcgctcatttcttttttattgctaaatactatgccactgtctggatgtgtcacagtttatttattcacctactgaaggacatcttgcttgtttccaagttgtggcaattgcgaattaagctgctacagacacccatgtgtgggtttttgtgtggacatgtttaccccacacaatttttaaagttgctcaa

SEQ ID NO: 3 - DNA, 19 bp, synthetic construct
  source 1..19: mol_type = other DNA
ccctgatgggagccagtgt

SEQ ID NO: 4 - DNA, 19 bp, synthetic construct
  source 1..19: mol_type = other DNA
agcagggagaagcccttca

SEQ ID NO: 5 - DNA, 27 bp, synthetic construct
  source 1..27: mol_type = other DNA
ccctggctttcaacacctacgtccact

SEQ ID NO: 6 - DNA, 20 bp, synthetic construct
  source 1..20: mol_type = other DNA
ggacaaggtggagggtctca

SEQ ID NO: 7 - DNA, 21 bp, synthetic construct
  source 1..21: mol_type = other DNA
agatccttgcagcaccagttg

SEQ ID NO: 8 - DNA, 29 bp, synthetic construct
  source 1..29: mol_type = other DNA
atgaagaaactatctccccggaccatcca

SEQ ID NO: 9 - DNA, 19 bp, synthetic construct
  source 1..19: mol_type = other DNA
gaaggtgaaggtcggagtc

SEQ ID NO: 10 - DNA, 20 bp, synthetic construct
  source 1..20: mol_type = other DNA
gaagatggtgatgggatttc

SEQ ID NO: 11 - DNA, 20 bp, synthetic construct
  source 1..20: mol_type = other DNA
caagcttcccgttctcagcc

SEQ ID NO: 12 - DNA, 16 bp, synthetic construct
  source 1..16: mol_type = other DNA
cgctgatttgtccggg

SEQ ID NO: 13 - DNA, 16 bp, synthetic construct
  source 1..16: mol_type = other DNA
tcggttggaattcttt

SEQ ID NO: 14 - DNA, 16 bp, synthetic construct
  source 1..16: mol_type = other DNA
  modified_base 14: mod_base = OTHER; note = uracil
tcggttggaattcttt

SEQ ID NO: 15 - DNA, 16 bp, synthetic construct
  source 1..16: mol_type = other DNA
gtcggttggaattctt

SEQ ID NO: 16 - DNA, 16 bp, synthetic construct
  source 1..16: mol_type = other DNA
  modified_base 6: mod_base = OTHER; note = uracil
ctcattgtggatgacg

SEQ ID NO: 17 - DNA, 16 bp, synthetic construct
  source 1..16: mol_type = other DNA
ctcattgtggatgacg

SEQ ID NO: 18 - DNA, 16 bp, synthetic construct
  source 1..16: mol_type = other DNA
  modified_base 6: mod_base = OTHER; note = uracil
tgaattggagcaggta

SEQ ID NO: 19 - DNA, 16 bp, synthetic construct
  source 1..16: mol_type = other DNA
tgaattggagcaggta

SEQ ID NO: 20 - DNA, 16 bp, synthetic construct
  source 1..16: mol_type = other DNA
cggtgtcaagttttgc

SEQ ID NO: 21 - DNA, 16 bp, synthetic construct
  source 1..16: mol_type = other DNA
gttgggtagactctgt

SEQ ID NO: 22 - DNA, 16 bp, synthetic construct
  source 1..16: mol_type = other DNA
gttggaattctttttg

SEQ ID NO: 23 - DNA, 16 bp, synthetic construct
  source 1..16: mol_type = other DNA
gttaagctgttgggta

SEQ ID NO: 24 - DNA, 16 bp, synthetic construct
  source 1..16: mol_type = other DNA
  modified_base 5: mod_base = OTHER; note = uracil
tgaattggagcaggta

SEQ ID NO: 25 - DNA, 16 bp, synthetic construct
  source 1..16: mol_type = other DNA
ttgcaggttcagctcg

SEQ ID NO: 26 - DNA, 16 bp, synthetic construct
  source 1..16: mol_type = other DNA
ggtagactctgtgggc

SEQ ID NO: 27 - DNA, 16 bp, synthetic construct
  source 1..16: mol_type = other DNA
gttggaattctttttg

SEQ ID NO: 28 - DNA, 20 bp, synthetic construct
  source 1..20: mol_type = other DNA
cacaaacaagctggtcggtt

SEQ ID NO: 29 - DNA, 16 bp, synthetic construct
  source 1..16: mol_type = other DNA
  modified_base 1: mod_base = OTHER; note = 2'-O-methoxyethyl 5-methylcytidine 3'-phosphorothioate
  modified_base 2: mod_base = OTHER; note = 2'-O-methoxyethyl guanosine 3'-phosphodiester
  modified_base 3: mod_base = OTHER; note = constrained ethyl 5-methylcytidine 3'-phosphodiester
  modified_base 4: mod_base = OTHER; note = 2'-deoxythymidine 3'-phosphorothioate
  modified_base 5: mod_base = OTHER; note = 2'-deoxyguanosine 3'-phosphorothioate
  modified_base 6: mod_base = OTHER; note = 2'-deoxyadenosine 3'-phosphorothioate
  modified_base 7..9: mod_base = OTHER; note = 2'-deoxythymidine 3'-phosphorothioate
  modified_base 10: mod_base = OTHER; note = 2'-deoxyguanosine 3'-phosphorothioate
  modified_base 11: mod_base = OTHER; note = 2'-deoxythymidine 3'-phosphorothioate
  modified_base 12..13: mod_base = OTHER; note = 5-methyl-2'-deoxycytidine 3'-phosphorothioate
  modified_base 14: mod_base = OTHER; note = constrained ethyl guanosine 3'-phosphodiester
  modified_base 15: mod_base = OTHER; note = constrained ethyl guanosine 3'-phosphorothioate
  modified_base 16: mod_base = OTHER; note = 2'-O-methoxyethyl guanosine
cgctgatttgtccggg

SEQ ID NO: 30 - DNA, 16 bp, synthetic construct
  source 1..16: mol_type = other DNA
  modified_base 1: mod_base = OTHER; note = 2'-O-methoxyethyl thymidine 3'-phosphorothioate
  modified_base 2: mod_base = OTHER; note = constrained ethyl 5-methylcytidine 3'-phosphodiester
  modified_base 3: mod_base = OTHER; note = constrained ethyl guanosine 3'-phosphodiester
  modified_base 4: mod_base = OTHER; note = 2'-deoxyguanosine 3'-phosphorothioate
  modified_base 5..6: mod_base = OTHER; note = 2'-deoxythymidine 3'-phosphorothioate
  modified_base 7..8: mod_base = OTHER; note = 2'-deoxyguanosine 3'-phosphorothioate
  modified_base 9..10: mod_base = OTHER; note = 2'-deoxyadenosine 3'-phosphorothioate
  modified_base 11..12: mod_base = OTHER; note = 2'-deoxythymidine 3'-phosphorothioate
  modified_base 13: mod_base = OTHER; note = 5-methyl-2'-deoxycytidine 3'-phosphorothioate
  modified_base 14: mod_base = OTHER; note = constrained ethyl thymidine 3'-phosphodiester
  modified_base 15: mod_base = OTHER; note = constrained ethyl thymidine 3'-phosphorothioate
  modified_base 16: mod_base = OTHER; note = 2'-O-methoxyethyl thymidine
tcggttggaattcttt

SEQ ID NO: 31 - DNA, 16 bp, synthetic construct
  source 1..16: mol_type = other DNA
  modified_base 5: mod_base = OTHER; note = uracil
  modified_base 1: mod_base = OTHER; note = constrained ethyl thymidine 3'-phosphorothioate
  modified_base 2: mod_base = OTHER; note = constrained ethyl 5-methylcytidine 3'-phosphodiester
  modified_base 3: mod_base = OTHER; note = constrained ethyl guanosine 3'-phosphodiester
  modified_base 4: mod_base = OTHER; note = 2'-deoxyguanosine 3'-phosphorothioate
  modified_base 5: mod_base = OTHER; note = 2'-O-methyl uridine 3'-phosphorothioate
  modified_base 6: mod_base = OTHER; note = 2'-deoxythymidine 3'-phosphorothioate
  modified_base 7..8: mod_base = OTHER; note = 2'-deoxyguanosine 3'-phosphorothioate
  modified_base 9..10: mod_base = OTHER; note = 2'-deoxyadenosine 3'-phosphorothioate
  modified_base 11..12: mod_base = OTHER; note = 2'-deoxythymidine 3'-phosphorothioate
  modified_base 13: mod_base = OTHER; note = 5-methyl-2'-deoxycytidine 3'-phosphorothioate
  modified_base 14: mod_base = OTHER; note = constrained ethyl thymidine 3'-phosphodiester
  modified_base 15: mod_base = OTHER; note = constrained ethyl thymidine 3'-phosphorothioate
  modified_base 16: mod_base = OTHER; note = constrained ethyl thymidine
tcggttggaattcttt

SEQ ID NO: 32 - DNA, 16 bp, synthetic construct
  source 1..16: mol_type = other DNA
  modified_base 1: mod_base = OTHER; note = constrained ethyl guanosine 3'-phosphorothioate
  modified_base 2: mod_base = OTHER; note = constrained ethyl thymidine 3'-phosphorothioate
  modified_base 3: mod_base = OTHER; note = constrained ethyl 5-methylcytidine 3'-phosphorothioate
  modified_base 4: mod_base = OTHER; note = 2'-deoxyguanosine 3'-phosphorothioate
  modified_base 5: mod_base = OTHER; note = 2'-O-methyl guanosine 3'-phosphorothioate
  modified_base 6..7: mod_base = OTHER; note = 2'-deoxythymidine 3'-phosphorothioate
  modified_base 8..9: mod_base = OTHER; note = 2'-deoxyguanosine 3'-phosphorothioate
  modified_base 10..11: mod_base = OTHER; note = 2'-deoxyadenosine 3'-phosphorothioate
  modified_base 12..13: mod_base = OTHER; note = 2'-deoxythymidine 3'-phosphorothioate
  modified_base 14: mod_base = OTHER; note = constrained ethyl 5-methylcytidine 3'-phosphorothioate
  modified_base 15: mod_base = OTHER; note = constrained ethyl thymidine 3'-phosphorothioate
  modified_base 16: mod_base = OTHER; note = constrained ethyl thymidine
gtcggttggaattctt

SEQ ID NO: 33 - DNA, 16 bp, synthetic construct
  source 1..16: mol_type = other DNA
  modified_base <1: mod_base = OTHER; note = Trishexylamino-N-Acetylgalactosamine-6-aminohexyl phosphodiester
  modified_base 1: mod_base = OTHER; note = 2'-O-methoxyethyl 5-methylcytidine 3'-phosphorothioate
  modified_base 2: mod_base = OTHER; note = 2'-O-methoxyethyl guanosine 3'-phosphodiester
  modified_base 3: mod_base = OTHER; note = constrained ethyl 5-methylcytidine 3'-phosphodiester
  modified_base 4: mod_base = OTHER; note = 2'-deoxythymidine 3'-phosphorothioate
  modified_base 5: mod_base = OTHER; note = 2'-deoxyguanosine 3'-phosphorothioate
  modified_base 6: mod_base = OTHER; note = 2'-deoxyadenosine 3'-phosphorothioate
  modified_base 7..9: mod_base = OTHER; note = 2'-deoxythymidine 3'-phosphorothioate
  modified_base 10: mod_base = OTHER; note = 2'-deoxyguanosine 3'-phosphorothioate
  modified_base 11: mod_base = OTHER; note = 2'-deoxythymidine 3'-phosphorothioate
  modified_base 12..13: mod_base = OTHER; note = 5-methyl-2'-deoxycytidine 3'-phosphorothioate
  modified_base 14: mod_base = OTHER; note = constrained ethyl guanosine 3'-phosphodiester
  modified_base 15: mod_base = OTHER; note = constrained ethyl guanosine 3'-phosphorothioate
  modified_base 16: mod_base = OTHER; note = 2'-O-methoxyethyl guanosine
cgctgatttgtccggg

SEQ ID NO: 34 - DNA, 16 bp, synthetic construct
  source 1..16: mol_type = other DNA
  modified_base <1: mod_base = OTHER; note = Trishexylamino-N-Acetylgalactosamine-6-aminohexyl phosphodiester
  modified_base 1: mod_base = OTHER; note = 2'-O-methoxyethyl thymidine 3'-phosphorothioate
  modified_base 2: mod_base = OTHER; note = constrained ethyl 5-methylcytidine 3'-phosphodiester
  modified_base 3: mod_base = OTHER; note = constrained ethyl guanosine 3'-phosphodiester
  modified_base 4: mod_base = OTHER; note = 2'-deoxyguanosine 3'-phosphorothioate
  modified_base 5..6: mod_base = OTHER; note = 2'-deoxythymidine 3'-phosphorothioate
  modified_base 7..8: mod_base = OTHER; note = 2'-deoxyguanosine 3'-phosphorothioate
  modified_base 9..10: mod_base = OTHER; note = 2'-deoxyadenosine 3'-phosphorothioate
  modified_base 11..12: mod_base = OTHER; note = 2'-deoxythymidine 3'-phosphorothioate
  modified_base 13: mod_base = OTHER; note = 5-methyl-2'-deoxycytidine 3'-phosphorothioate
  modified_base 14: mod_base = OTHER; note = constrained ethyl thymidine 3'-phosphodiester
  modified_base 15: mod_base = OTHER; note = constrained ethyl thymidine 3'-phosphorothioate
  modified_base 16: mod_base = OTHER; note = 2'-O-methoxyethyl thymidine
tcggttggaattcttt

SEQ ID NO: 35 - DNA, 16 bp, synthetic construct
  source 1..16: mol_type = other DNA
  modified_base 5: mod_base = OTHER; note = uracil
  modified_base <1: mod_base = OTHER; note = Trishexylamino-N-Acetylgalactosamine-6-aminohexyl phosphodiester
  modified_base 1: mod_base = OTHER; note = constrained ethyl thymidine 3'-phosphorothioate
  modified_base 2: mod_base = OTHER; note = constrained ethyl 5-methylcytidine 3'-phosphodiester
  modified_base 3: mod_base = OTHER; note = constrained ethyl guanosine 3'-phosphodiester
  modified_base 4: mod_base = OTHER; note = 2'-deoxyguanosine 3'-phosphorothioate
  modified_base 5: mod_base = OTHER; note = 2'-O-methyl uridine 3'-phosphorothioate
  modified_base 6: mod_base = OTHER; note = 2'-deoxythymidine 3'-phosphorothioate
  modified_base 7..8: mod_base = OTHER; note = 2'-deoxyguanosine 3'-phosphorothioate
  modified_base 9..10: mod_base = OTHER; note = 2'-deoxyadenosine 3'-phosphorothioate
  modified_base 11..12: mod_base = OTHER; note = 2'-deoxythymidine 3'-phosphorothioate
  modified_base 13: mod_base = OTHER; note = 5-methyl-2'-deoxycytidine 3'-phosphorothioate
  modified_base 14: mod_base = OTHER; note = constrained ethyl thymidine 3'-phosphodiester
  modified_base 15: mod_base = OTHER; note = constrained ethyl thymidine 3'-phosphorothioate
  modified_base 16: mod_base = OTHER; note = constrained ethyl thymidine
tcggttggaattcttt

SEQ ID NO: 36 - DNA, 16 bp, synthetic construct
  source 1..16: mol_type = other DNA
  modified_base <1: mod_base = OTHER; note = Trishexylamino-N-Acetylgalactosamine-6-aminohexyl phosphodiester
  modified_base 1: mod_base = OTHER; note = constrained ethyl guanosine 3'-phosphorothioate
  modified_base 2: mod_base = OTHER; note = constrained ethyl thymidine 3'-phosphorothioate
  modified_base 3: mod_base = OTHER; note = constrained ethyl 5-methylcytidine 3'-phosphorothioate
  modified_base 4: mod_base = OTHER; note = 2'-deoxyguanosine 3'-phosphorothioate
  modified_base 5: mod_base = OTHER; note = 2'-O-methyl guanosine 3'-phosphorothioate
  modified_base 6..7: mod_base = OTHER; note = 2'-deoxythymidine 3'-phosphorothioate
  modified_base 8..9: mod_base = OTHER; note = 2'-deoxyguanosine 3'-phosphorothioate
  modified_base 10..11: mod_base = OTHER; note = 2'-deoxyadenosine 3'-phosphorothioate
  modified_base 12..13: mod_base = OTHER; note = 2'-deoxythymidine 3'-phosphorothioate
  modified_base 14: mod_base = OTHER; note = constrained ethyl 5-methylcytidine 3'-phosphorothioate
  modified_base 15: mod_base = OTHER; note = constrained ethyl thymidine 3'-phosphorothioate
  modified_base 16: mod_base = OTHER; note = constrained ethyl thymidine
gtcggttggaattctt